European Patent Specification EP 3 867 640 B9, published October 4, 2023. Title: Method for identifying a chemical compound or agent inducing ubiquitination of a protein of interest. Applicant: CeMM - Forschungszentrum für Molekulare Medizin GmbH. The sequence listing filed with the application follows.

SEQUENCE LISTING (5 sequences)

SEQ ID NO: 1 - RNA, 20 nt, Artificial Sequence
  Primer
ccggttgctccggaagtgga

SEQ ID NO: 2 - DNA, 120 bp, Artificial Sequence
  Oligonucleotide
aggggccggttgctccggaagtgccaccatggtgagcggctggcggctgttcaagaagattagcggctatccgtatgatgtcccggactatgcaaggagggagggggtgaaaatggcgcc

SEQ ID NO: 3 - protein, 12 aa, Artificial Sequence
  Hibit sequence
MVSGWRLFKKIS

SEQ ID NO: 4 - protein, 9 aa, Artificial Sequence
  HA-sequence
YPYDVPDYA

SEQ ID NO: 5 - protein, 30 aa, Artificial Sequence
  Hibit-HA-MH sequence
MVSGWRLFKKISGYPYDVPDYARREGVKMA